European Patent Application EP 4 364 740 A1, published May 8, 2024. Title: A pharmaceutical composition for preventing or treating cancer. Applicant: Industry-Academic Cooperation Foundation, Yonsei University. The sequence listing filed with the application follows.

SEQUENCE LISTING (5 sequences)

SEQ ID NO: 1 - RNA, 2010 nt, Homo sapiens
atgatgcggctgcgaggctcggggatgctgcgggacctgctcctgcggtcgcccgccggcgtgagcgcgactctgcggcgggcacagcccttggtcaccctgtgccggcgtccccgaggcgggggacggccggccgcgggcccggctgccgccgcgcgactccacccgtggtggggcgggggcggctggccggcggagcccctcgcgcggggcctgtccagctctccttcggagatcttgcaggagctgggcaaggggagcacgcatccgcagcccggggtgtcgccacccgctgccccggcggcgcccggccccaaggacggccccggggagacggacgcgtttggcaacagcgagggcaaagagctggtggcctcaggtgaaaataaaataaaacagggtctgttacctagcttggaagatttgctgttctatacaattgctgaaggacaagagaaaatacctgttcataaatttattacagcactcaaatctacaggattgcgaacgtctgatcccaggttgaaagagtgtatggatatgttaagattaactcttcaaacaacatcagatggtgtcatgctagacaaagatctttttaaaaaatgtgttcagagcaacattgttttgttgacacaagcatttagaagaaagtttgtgattcctgactttatgtcttttacctcacacattgatgagttatatgaaagtgctaaaaagcagtctggaggaaaggttgcagattatattcctcaactggccaaattcagtcccgatttgtggggtgtgtctgtttgtacagtagatggacagaggcattctactggagataccaaagttcccttctgtcttcagtcctgtgtaaaacctttgaaatatgccattgctgttaatgatcttggaactgaatatgtgcatcgatatgttggaaaagagccgagtggactaagattcaacaaactatttttgaatgaagatgataaaccacataatcctatggtaaatgctggagcaattgttgtgacttcactaataaagcaaggagtaaataatgctgaaaaatttgactatgtcatgcagtttttgaataagatggctggtaatgaatatgttggattcagtaatgcaacgtttcagtctgaaagagaaagtggagatcgaaattttgcaataggatattacttaaaagaaaagaagtgttttccagaaggcacagacatggttggtatattagacttctacttccagctgtgctccattgaagtgacttgtgaatcagccagtgtgatggctgcgacactggctaatggtggtttctgcccaattactggtgaaagagtactgagccctgaagcagttcgaaatacattgagtttgatgcattcctgtggcatgtatgacttctcagggcagtttgctttccatgttggtcttcctgcaaaatctggagttgctgggggcattcttttagttgtccccaatgttatgggtatgatgtgctggtctcctcctctggataagatgggcaacagtgttaagggaattcacttttgtcacgatcttgtttctctgtgtaatttccataactatgataatttgagacactttgcaaaaaaacttgatcctcgaagagaaggtggtgatcaaagggtaaagtcagtgataaatcttttgtttgctgcatatactggagatgtgtctgcacttcgaagatttgctttgtcagctatggacatggaacagcgggactatgattctagaacagcactccatgtagctgctgcagagggtcatgttgaagttgttaaatttttgctggaagcctgcaaagtaaaccctttccccaaggacaggtggaataacactcccatggatgaagcactgcactttggacaccatgatgtatttaaaattctccaagaataccaagtccagtacacacctcaaggagattctgacaacgggaaggaaaatcaaaccgtccataagaatcttgatggattgttgtaa

SEQ ID NO: 2 - RNA, 1797 nt, Homo sapiens
atgatgcggctgcgaggctcggggatgctgcgggacctgctcctgcggtcgcccgccggcgtgagcgcgactctgcggcgggcacagcccttggtcaccctgtgccggcgtccccgaggcgggggacggccggccgcgggcccggctgccgccgcgcgactccacccgtggtggggcgggggcggctggccggcggagcccctcgcgcggggcctgtccagctctccttcggagatcttgcaggagctgggcaaggggagcacgcatccgcagcccggggtgtcgccacccgctgccccggcggcgcccggccccaaggacggccccggggagacggacgcgtttggcaacagcgagggcaaagagctggtggcctcaggtgaaaataaaataaaacagggtctgttacctagcttggaagatttgctgttctatacaattgctgaaggacaagagaaaatacctgttcataaatttattacagcactcaaatctacaggattgcgaacgtctgatcccaggttgaaagagtgtatggatatgttaagattaactcttcaaacaacatcagatggtgtcatgctagacaaagatctttttaaaaaatgtgttcagagcaacattgttttgttgacacaagcatttagaagaaagtttgtgattcctgactttatgtcttttacctcacacattgatgagttatatgaaagtgctaaaaagcagtctggaggaaaggttgcagattatattcctcaactggccaaattcagtcccgatttgtggggtgtgtctgtttgtacagtagatggacagaggcattctactggagataccaaagttcccttctgtcttcagtcctgtgtaaaacctttgaaatatgccattgctgttaatgatcttggaactgaatatgtgcatcgatatgttggaaaagagccgagtggactaagattcaacaaactatttttgaatgaagatgataaaccacataatcctatggtaaatgctggagcaattgttgtgacttcactaataaagcaaggagtaaataatgctgaaaaatttgactatgtcatgcagtttttgaataagatggctggtaatgaatatgttggattcagtaatgcaacgtttcagtctgaaagagaaagtggagatcgaaattttgcaataggatattacttaaaagaaaagaagtgttttccagaaggcacagacatggttggtatattagacttctacttccagctgtgctccattgaagtgacttgtgaatcagccagtgtgatggctgcgacactggctaatggtggtttctgcccaattactggtgaaagagtactgagccctgaagcagttcgaaatacattgagtttgatgcattcctgtggcatgtatgacttctcagggcagtttgctttccatgttggtcttcctgcaaaatctggagttgctgggggcattcttttagttgtccccaatgttatgggtatgatgtgctggtctcctcctctggataagatgggcaacagtgttaagggaattcacttttgtcacgatcttgtttctctgtgtaatttccataactatgataatttgagacactttgcaaaaaaacttgatcctcgaagagaaggtggtgatcaaaggcattcctttggaccattggactatgaaagtctccaacaagaacttgctttaaaagagacagtatggaaaaaagtgtcacctgagtcaaatgaggacatctctacaactgtagtatatagaatggaaagtctgggagagaaaagctaa

SEQ ID NO: 3 - RNA, 1602 nt, Homo sapiens
atggcttttgcaaatctgcggaaagtgctcatcagtgacagcctggacccttgctgccggaagatcttgcaagatggagggctgcaggtggtggaaaagcagaaccttagcaaagaggagctgatagcggagctgcaggactgtgaaggccttattgttcgctctgccaccaaggtgaccgctgatgtcatcaacgcagctgagaaactccaggtggtgggcagggctggcacaggtgtggacaatgtggatctggaggccgcaacaaggaagggcatcttggttatgaacacccccaatgggaacagcctcagtgccgcagaactcacttgtggaatgatcatgtgcctggccaggcagattccccaggcgacggcttcgatgaaggacggcaaatgggagcggaagaagttcatgggaacagagctgaatggaaagaccctgggaattcttggcctgggcaggattgggagagaggtagctacccggatgcagtcctttgggatgaagactatagggtatgaccccatcatttccccagaggtctcggcctcctttggtgttcagcagctgcccctggaggagatctggcctctctgtgatttcatcactgtgcacactcctctcctgccctccacgacaggcttgctgaatgacaacacctttgcccagtgcaagaagggggtgcgtgtggtgaactgtgcccgtggagggatcgtggacgaaggcgccctgctccgggccctgcagtctggccagtgtgccggggctgcactggacgtgtttacggaagagccgccacgggaccgggccttggtggaccatgagaatgtcatcagctgtccccacctgggtgccagcaccaaggaggctcagagccgctgtggggaggaaattgctgttcagttcgtggacatggtgaaggggaaatctctcacgggggttgtgaatgcccaggcccttaccagtgccttctctccacacaccaagccttggattggtctggcagaagctctggggacactgatgcgagcctgggctgggtcccccaaagggaccatccaggtgataacacagggaacatccctgaagaatgctgggaactgcctaagccccgcagtcattgtcggcctcctgaaagaggcttccaagcaggcggatgtgaacttggtgaacgctaagctgctggtgaaagaggctggcctcaatgtcaccacctcccacagccctgctgcaccaggggagcaaggcttcggggaatgcctcctggccgtggccctggcaggcgccccttaccaggctgtgggcttggtccaaggcactacacctgtactgcaggggctcaatggagctgtcttcaggccagaagtgcctctccgcagggacctgcccctgctcctattccggactcagacctctgaccctgcaatgctgcctaccatgattggcctcctggcagaggcaggcgtgcggctgctgtcctaccagacttcactggtgtcagatggggagacctggcacgtcatgggcatctcctccttgctgcccagcctggaagcgtggaagcagcatgtgactgaagccttccagttccacttctaa

SEQ ID NO: 4 - RNA, 1485 nt, Homo sapiens
atgctgtacttctctttgttttgggcggctcggcctctgcagagatgtgggcagctggtcaggatggccattcgggctcagcacagcaacgcagcccagactcagactggggaagcaaacaggggctggacaggccaggagagcctgtcggacagtgatcctgagatgtgggagttgctgcagagggagaaggacaggcagtgtcgtggcctggagctcattgcctcagagaacttctgcagccgagctgcgctggaggccctggggtcctgtctgaacaacaagtactcggagggttatcctggcaagagatactatgggggagcagaggtggtggatgaaattgagctgctgtgccagcgccgggccttggaagcctttgacctggatcctgcacagtggggagtcaatgtccagccctactccgggtccccagccaacctggccgtctacacagcccttctgcaacctcacgaccggatcatggggctggacctgcccgatgggggccatctcacccacggctacatgtctgacgtcaagcggatatcagccacgtccatcttcttcgagtctatgccctataagctcaacctggcactgactgctcgacttttccggccacggctcatcatagctggcaccagcgcctatgctcgcctcattgactacgcccgcatgagagaggtgtgtgatgaagtcaaagcacacctgctggcagacatggcccacatcagtggcctggtggctgccaaggtgattccctcgcctttcaagcacgcggacatcgtcaccaccactactcacaagactcttcgaggggccaggtcagggctcatcttctaccggaaaggggtgaaggctgtggaccccaagactggccgggagatcccttacacatttgaggaccgaatcaactttgccgtgttcccatccctgcaggggggcccccacaatcatgccattgctgcagtagctgtggccctaaagcaggcctgcacccccatgttccgggagtactccctgcaggttctgaagaatgctcgggccatggcagatgccctgctagagcgaggctactcactggtatcaggtggtactgacaaccacctggtgctggtggacctgcggcccaagggcctggatggagctcgggctgagcgggtgctagagcttgtatccatcactgccaacaagaacacctgtcctggagaccgaagtgccatcacaccgggcggcctgcggcttggggccccagccttaacttctcgacagttccgtgaggatgacttccggagagttgtggactttatagatgaaggggtcaacattggcttagaggtgaagagcaagactgccaagctccaggatttcaaatccttcctgcttaaggactcagaaacaagtcagcgtctggccaacctcaggcaacgggtggagcagtttgccagggccttccccatgcctggttttgatgagcattga

SEQ ID NO: 5 - RNA, 1053 nt, Homo sapiens
atggctgcgacttctctaatgtctgctttggctgcccggctgctgcagcccgcgcacagctgctcccttcgccttcgccctttccacctcgcggcagttcgaaatgaagctgttgtcatttctggaaggaaactggcccagcagatcaagcaggaagtgcggcaggaggtagaagagtgggtggcctcaggcaacaaacggccacacctgagtgtgatcctggttggcgagaatcctgcaagtcactcctatgtcctcaacaaaaccagggcagctgcagttgtgggaatcaacagtgagacaattatgaaaccagcttcaatttcagaggaagaattgttgaatttaatcaataaactgaataatgatgataatgtagatggcctccttgttcagttgcctcttccagagcatattgatgagagaaggatctgcaatgctgtttctccagacaaggatgttgatggctttcatgtaattaatgtaggacgaatgtgtttggatcagtattccatgttaccggctactccatggggtgtgtgggaaataatcaagcgaactggcattccaaccctagggaagaatgtggttgtggctggaaggtcaaaaaacgttggaatgcccattgcaatgttactgcacacagatggggcgcatgaacgtcccggaggtgatgccactgttacaatatctcatcgatatactcccaaagagcagttgaagaaacatacaattcttgcagatattgtaatatctgctgcaggtattccaaatctgatcacagcagatatgatcaaggaaggagcagcagtcattgatgtgggaataaatagagttcacgatcctgtaactgccaaacccaagttggttggagatgtggattttgaaggagtcagacaaaaagctgggtatatcactccagttcctggaggtgttggccccatgacagtggcaatgctaatgaagaataccattattgctgcaaaaaaggtgctgaggcttgaagagcgagaagtgctgaagtctaaagagcttggggtagccactaattaa